European Patent Application EP 4 289 859 A1, published December 13, 2023. Title: Fusion protein for maintenance of regulatory T-cells. Applicant: Medizinische Hochschule Hannover. The sequence listing filed with the application follows.

SEQUENCE LISTING (2 sequences)

SEQ ID NO: 1 - protein, 234 aa, Artificial Sequence
  SIGNAL 1..20: signal peptide
  IL-2 fusion protein
  CHAIN 21..153: IL-2
  CHAIN 154..177: linker
  CHAIN 178..201: transmembrane domain
  CHAIN 202..234: anchor
MYRMQLLSCIALSLALVTNSAPTSSSTKKTQLQLEHLLLDLQMILNGINNYKNPKLTRMLTFKFYMPKKATELKHLQCLEEELKPLEEVLNLAQSKNFHLRPRDLISNINVIVLELKGSETTFMCEYADETATIVEFLNRWITFCQSIISTLTRSGGGGSGGGSGGGSPSSQPTIPIVGIIAGLVLFGAVITGAVVAAVMWRRKSSDRKGGSYSQAASSDSAQGSDVSLTACKV

SEQ ID NO: 2 - protein, 768 aa, Artificial Sequence
  CHAIN 1..21: signal peptide
  Fusion protein including CAR and membrane-bound IL-2
  CHAIN 22..270: scFv
  CHAIN 273..354: hinge CD8
  CHAIN 357..399: CD28 signal domain
  CHAIN 400..512: CD3zeta signal domain
  CHAIN 515..533: P2A site
  CHAIN 535..554: IL-2 signal peptide
  CHAIN 555..687: IL-2
  CHAIN 688..702: GS linker section
  CHAIN 703..711: 8 amino acid plus proline linker section
  CHAIN 712..735: transmembrane domain
  CHAIN 736..768: anchor domain
MWWRLWWLLLLLLLLWPMVWAMAQVQLVQSGGGVVQPGGSLRVSCAASGVTLSDYGMHWVRQAPGKGLEWVAFIRNDGSDKYYADSVKGRFTISRDNSEKTVSLQMSSLRAEDTAVYYCAKNGESGPLDYWYLDLWGRGTLVTVSSGGGGSGGGGSGGGGSTDVVMTQSPSSLSASVGDRVTITCQSSLDISHYLNWYQQKPGKAPKLLIYDASNLETGVPSRFSGSGSGTHFTFTISSLQPEDFATYYCQQYDNLPLTFGGGTKLEIKRAAAFVPVFLPAKPTTTPAPRPPTPAPTIASQPLSLRPEASRPAAGGAVHTRGLDFADIYIWAPLAGTCGVLLLSLVITLYCNHRQLWVRSKRSRLLHSDYMNMTPRRPGPTRKHYQPYAPPRDFAAYRSRVKFSRSADAPAYQQGQNQLYNELNLGRREEYDVLDKRRGRDPEMGGKPRRKNPQEGLYNELQKDKMAEAYSEIGMKGERRRGKGHDGLYQGLSTATKDTYDALHMQALPPRSSRATNFSLLKQAGDVEENPGPSMYRMQLLSCIALSLALVTNSAPTSSSTKKTQLQLEHLLLDLQMILNGINNYKNPKLTRMLTFKFYMPKKATELKHLQCLEEELKPLEEVLNLAQSKNFHLRPRDLISNINVIVLELKGSETTFMCEYADETATIVEFLNRWITFCQSIISTLTRSGGGGSGGGSGGGSPSSQPTIPIVGIIAGLVLFGAVITGAVVAAVMWRRKSSDRKGGSYSQAASSDSAQGSDVSLTACKV